European Patent Application EP 4 335 926 A2, published March 13, 2024. Title: NANOS KNOCKOUT THAT ABLATES GERMLINE CELLS. Applicant: Washington State University. The sequence listing filed with the application follows.

SEQUENCE LISTING (204 sequences)

SEQ ID NO: 1 - DNA, 417 bp, Sus scrofa
  source 1..417: mol_type = other DNA
atgcagctgccaccctttgacatgtggaaggactacttcaacctgagccaggtggtgttgggactgatccagaatcgtcgacaagggccagaggccccgggcaccggggagccaagacctgagcccccactggagcaggaccagggcccgggagagcggggggccagcggggggctggccaccctgtgcaacttttgcaaacacaatggggaatctcgccacgtgtactcctcgcaccagctgaagacaccggagggcgtggtggtgtgtcccatcctacgacactatgtgtgtcccctgtgcggggccaccggtgaccaggctcacacactcaagtactgcccgctcaacggcggccagcagtctctctatcgccgcagtgggcgcaattcagccggccgcaaggtcaagcgctga

SEQ ID NO: 2 - protein, 138 aa, Sus scrofa
MQLPPFDMWKDYFNLSQVVLGLIQNRRQGPEAPGTGEPRPEPPLEQDQGPGERGASGGLATLCNFCKHNGESRHVYSSHQLKTPEGVVVCPILRHYVCPLCGATGDQAHTLKYCPLNGGQQSLYRRSGRNSAGRKVKR

SEQ ID NO: 3 - DNA, 1073 bp, Sus scrofa
  source 1..1073: mol_type = other DNA
cagcccacccagggaccatgcattcctttggcaggtgcatttttggaggagcagcagcaagcccccctgtgacaataaggaacctcccacagcctgctcctccctcttcacacccccttggaggtataaggagggaactgacagcccagactcctgggctccagagagagaaagggaggggcagggggaaggggatagaaggacgatctttggggtggctgggtttcttctctctctctgccctttcacctggtacactttgcccagccatggggaccttcaacctgtggacagattacctgggtttggcacgcctggtgggggctctgcgtggggaagaggaacctgagacgaggctggacccccagccagcaccagtgccaggaccagagggtcagaggcccagcccggaatcctcaccagctcctgaacgcctgtgctctttctgcaaacataatggcgaatcccgggccatctaccagtcccacgtgctcaaggatgaagcgggccgagttctgtgccccattcttcgagactacgtgtgcccccagtgcggtgccacacgcgagcgtgcccatacccgccgcttctgccctctcaccagccagggctacacctctgtctacagctacaccacccgcaactcggccggcaagaagctggcccgcccggacaaggcgaggacacaggactctggacatcggcgaggaggaggaggaggaggtgccagcacaggttccaaaggtgccgggaagtcttctggaacttctccgtctccctgctgtccctccacttctgcctaagaggctggcgcgagcaggacggagatgctgccttcacctggggatggggacccaggctcagtggaggctgggtttcagggacgacctacccttcgcggatccgcccctgcccccagcctgggagccctgcaagggagccaggcctggaagctcggccaaaagagagccgctcctttctccccatctcccaccccaagaaaggaggtggtcctctggcaaccctgccctccttccccagcgctgggcacccagttagcactcaataaatac

SEQ ID NO: 4 - protein, 261 aa, Sus scrofa
MHSFGRCIFGGAAASPPVTIRNLPQPAPPSSHPLGGIRRELTAQTPGLQREKGRGRGKGIEGRSLGWLGFFSLSALSPGTLCPAMGTFNLWTDYLGLARLVGALRGEEEPETRLDPQPAPVPGPEGQRPSPESSPAPERLCSFCKHNGESRAIYQSHVLKDEAGRVLCPILRDYVCPQCGATRERAHTRRFCPLTSQGYTSVYSYTTRNSAGKKLARPDKARTQDSGHRRGGGGGGASTGSKGAGKSSGTSPSPCCPSTSA

SEQ ID NO: 5 - DNA, 1906 bp, Sus scrofa
  source 1..1906: mol_type = other DNA
cgcagggggcagggccgcggcagcgaggccggggggcggggaggagcggggcccgataaaaggcagcgaggcggccccaccccgctgcaggccggcgggcaggctcggcgcgtcctttccgtccggcccgcgccggcggcggggaggcggcgcgcgcggcccgcagcccgcccatggaggctttcccctgggcgccccgctcgccccgccgcggccgcgtccccccgcccatggcgctcgtgcccagcgcccgctacgtgagcgcccagggcccggcgcacccgcaacccttcagctcgtggaacgactacctgggactcgccacgctcatcaccaaggcggtggacggcgagccgcgctttggctgcgcccgcggcgaggacggcggcggcggcggcggctccccaccctcctcttcctcctcgtcgtgctgctccccccacgcgggggccgggcctggggcgctggggcccgcgctggggccacccgactacgacgaggacgacgacgacgacagcgacgagccggggtcccggggccgctacctggggggcacgctggagctgcgcgcgctggagctgtgcgcggacccctcggaggccgggctgctggaggagcgcttcgccgagctgagcccgttcgcgggtcgcgccaccgctgtgctgctgggctgggcacccgccactgccgccaccgccgaggcggcaccgcgcgaggagcgggccccggcgtgggcggccgagccccggctgcacgcagcctttggggcggccggcgcccggctgctcaagcccgagctgcaggtgtgtgtgttttgccggaacaacaaggaggcggtggcgctctacaccacccacatcttgaagggacccgacgggcgagtgctgtgccccgtgctgcgccgctacacgtgtcccctgtgcggcgccagcggcgacaacgcgcacaccatcaagtactgcccgctctccaaagtgccgccgccgcgcagcgtcagggacggcctgcccggcaagaagctgcgctgagggcccggactccggtctgctactgccacctgacgccaccagggtcgccgcctgcccaatgtctagtttggcctgcgcaccatctctctctctcgctgctgaggagcgtggagctcagctgttggttgaacttgagatgtactgattttttttttttttttttcaaaagaacccggcggtactgagtcctttcctgtcgaagagcgcttaagactagaagctaaaatcttgatttgtttatctctagtttgtgcacatccagacggtgaaggctgggtgttcgttccactaactgaaatgtggcaacttagaagtgtttatttactctatacgtcaacctattttagatgcgcatcagtatatgaaattgtctcaatctaatcttggatgtttaattttatgaatggaggcactttactaggcctagaatatttttttaaaagcctctaaactgaacttaactggcgattttatggaatgtcagcaaaatgacttttattgtttgaaacaagtaataatatttctgttgtccttaatcagttattctaattccaggtgaagcaaccctcacctgcctggtagcatcattaagtgaaggcttagtaaactttccagtgttagtttgggtgggtgttccccccgtggcttgtttctgtcctagctggaggtgtaaagatgtacaatctgtggcaggtagaatacagctccttatccttttatgtaccacatcttttattactgaacgagcaactagcgtttcccatctttcaaagtcgtgccaggttatataatattgtgtatacacttggaaatggtgctgtttaaaagaatttgtgtatttatacagtaacagtatatgaattcattaatcttgtctt

SEQ ID NO: 6 - protein, 284 aa, Sus scrofa
MEAFPWAPRSPRRGRVPPPMALVPSARYVSAQGPAHPQPFSSWNDYLGLATLITKAVDGEPRFGCARGEDGGGGGGSPPSSSSSSCCSPHAGAGPGALGPALGPPDYDEDDDDDSDEPGSRGRYLGGTLELRALELCADPSEAGLLEERFAELSPFAGRATAVLLGWAPATAATAEAAPREERAPAWAAEPRLHAAFGAAGARLLKPELQVCVFCRNNKEAVALYTTHILKGPDGRVLCPVLRRYTCPLCGASGDNAHTIKYCPLSKVPPPRSVRDGLPGKKLR

SEQ ID NO: 7 - DNA, 23 bp, Sus scrofa
  source 1..23: mol_type = other DNA
gaagacaccggagggcgtggtgg

SEQ ID NO: 8 - DNA, 23 bp, Sus scrofa
  source 1..23: mol_type = other DNA
gaatcgtcgacaagggccagagg

SEQ ID NO: 9 - DNA, 548 bp, Bos taurus
  source 1..548: mol_type = other DNA
tcagctgctcctgtctgcgggcccccagcccacttctctccagccacccaccaccaacactcccccgggtgccatgcagctgccaccctttgacatgtggaaggactacttcaacctgagccaagtggtgctggcactgatccagagtcgggggcaagggttggagacccaagggactggggagccgagacccgggccccatgtggagcaggatcaggggcagggcggacgcggggctggcgggggcctggccaccctgtgcaacttttgcaaacacaatggagagtctcgccacgtgtactcctcacaccagctgaagaccccggagggcgtggtggtgtgtcccattctgcggcattatgtatgtcccctgtgcggggccaccggggaccaggcccacacactcaagtactgcccactcaacggaggacagcagtctctctaccgccgcagtgggcgcaactcagccggccgcaaggtcaagcgctgaagaccgtcaggtacccacccgctgcagccccaaccctccctggttcagccctcccaag

SEQ ID NO: 10 - protein, 138 aa, Bos taurus
MQLPPFDMWKDYFNLSQVVLALIQSRGQGLETQGTGEPRPGPHVEQDQGQGGRGAGGGLATLCNFCKHNGESRHVYSSHQLKTPEGVVVCPILRHYVCPLCGATGDQAHTLKYCPLNGGQQSLYRRSGRNSAGRKVKR

SEQ ID NO: 11 - DNA, 1624 bp, Bos taurus
  source 1..1624: mol_type = other DNA
gccgccgccgcggccaccgccgaagcagcaccgcgagaggagcgggccccggcgtgggcggccgagcccaagctgcacgccgcctccggggcggccgccgcccggctgctcaagcccgagctgcaggtgtgcgtgttttgccggaacaacaaggaggcggtggcgctctacaccacccacatcctgaagggacccgacgggcgggtgctgtgccccgtgctgcgccggtacacgtgtcccctgtgcggtgccagcggcgacaacgcgcacaccatcaagtactgcccgctttccaaagtgccgccgccgcctgcagcccgcccgccgccgcgcagcgcccgggacggcctgcccggcaagaagctgcgctaagggcccggaccccggtctgctgctgccacctgatgccactggggtagccgcccgcccactctcgtgtttggtctgcgcaccatctcttcctcgctgccggggagtgtggagctcgtcttggtttttccagaggaagccgacggtaccgagtattttcctaacgaagagcagttgagactagacgttaaaattttgattaatgtttctagtttgtgcacatccagatggtgaaggctgggtattccactaactgaaatgtggcaacttagaggcgctgtggtttatttatacgtcgacctattttagatgcgcatcagtatgaaattgtctcagtctaatcttggatgtttaattttatgaatggaggcactttactaggtctagaatatttttttaaaagcctctcaactgaacttaaaactggcgattttatggagtgtcagcaaaatgactattttattgtctgaaacaatatttctgttgtccttacccagttgtaattccaggtgaagccctgcgtggtagcatcattaagtgaagacttggtatgctttacagtgttagtttgggtgggtgttccctccttgtggcttgtttttgtcctagctggagatgtataaaatgtacaatttgtaggtagcaggtagaatacagctcatgtaccagatctttttattactgaacgagcaactactaccgtttttcccctttaaaaatagtgccaagttataatcatattgtgtatacacttgaaaatggtgctgtttaaaaaaattgtgtatttatacagtaacagtatatgaattcattaaccttgcctttaactctacttggctttttctttatgccccttcctattccagttcttcaaaaatatgtgatacttaagatcaaacgggtgcaataactcattcactctgaattgctccatttcagggtctctaaatagtggaaatctcattccagctgttgcctctcagactaaatgtaagatggaatcctttgagctctggaaggttaatgaaacaactggtgttcaggaaggttccactctggactgtgtcagctttaaaccatcacagaagtcctcaaaccagtataagtaccaattaaaggaactgactgggtgtagggggggtaacacaaggaacacagcctccatctattgtgttcccattctcattagaagacaacccttctggaatcccaccagttattttcatcggtgagattaaatctaatcttgggcaaa

SEQ ID NO: 12 - protein, 123 aa, Bos taurus
AAAAATAEAAPREERAPAWAAEPKLHAASGAAAARLLKPELQVCVFCRNNKEAVALYTTHILKGPDGRVLCPVLRRYTCPLCGASGDNAHTIKYCPLSKVPPPPAARPPPRSARDGLPGKKLR

SEQ ID NO: 13 - DNA, 2056 bp, Bos taurus
  source 1..2056: mol_type = other DNA
cgctacgtgagcacccagggcccggcgcacccgcagcccttcagctcgtggaacgactatctgggactcgccacgctcatcaccaaggcggtggacggcgagccgcgcttcggctgcgcccgcggcggggacggcggcggggacggctccccgccttcttcttcctcctcgtcgtgctgctccccccacgtgggggccgggcctggggcgctggggcccgcgctggggccgcccgactacgacgaggacgacgacgacgacgacagcgacgatccggggtcccggagccgctacctggggggcgcgctggagctgcgcgcgctggagctgtgcgcggaccctgccgaggccgggctgctggaggagcgtttcgctgagctgagcccgttcgctggtcgcgccgctgccgtgcttctgggctgcgcacccgccgccgccgccgcggccaccgccgaagcagcaccgcgagaggagcgggccccggcgtgggcggccgagcccaagctgcacgccgcctccggggcggccgccgcccggctgctcaagcccgagctgcaggtgtgcgtgttttgccggaacaacaaggaggcggtggcgctctacaccacccacatcctgaagggacccgacgggcgggtgctgtgccccgtgctgcgccggtacacgtgtcccctgtgcggtgccagcggcgacaacgcgcacaccatcaagtactgcccgctttccaaagtgccgccgccgcctgcagcccgcccgccgccgcgcagcgcccgggacggcctgcccggcaagaagctgcgctaagggcccggaccccggtctgctgctgccacctgatgccactggggtagccgcccgcccactctcgtgtttggtctgcgcaccatctcttcctcgctgccggggagtgtggagctcgtcttggtttttccagaggaagccgacggtaccgagtattttcctaacgaagagcagttgagactagacgttaaaattttgattaatgtttctagtttgtgcacatccagatggtgaaggctgggtattccactaactgaaatgtggcaacttagaggcgctgtggtttatttatacgtcgacctattttagatgcgcatcagtatgaaattgtctcagtctaatcttggatgtttaattttatgaatggaggcactttactaggtctagaatatttttttaaaagcctctcaactgaacttaaaactggcgattttatggagtgtcagcaaaatgactattttattgtctgaaacaatatttctgttgtccttacccagttgtaattccaggtgaagccctgcgtggtagcatcattaagtgaagacttggtatgctttacagtgttagtttgggtgggtgttccctccttgtggcttgtttttgtcctagctggagatgtataaaatgtacaatttgtaggtagcaggtagaatacagctcatgtaccagatctttttattactgaacgagcaactactaccgtttttcccctttaaaaatagtgccaagttataatcatattgtgtatacacttgaaaatggtgctgtttaaaaaaattgtgtatttatacagtaacagtatatgaattcattaaccttgcctttaactctacttggctttttctttatgccccttcctattccagttcttcaaaaatatgtgatacttaagatcaaacgggtgcaataactcattcactctgaattgctccatttcagggtctctaaatagtggaaatctcattccagctgttgcctctcagactaaatgtaagatggaatcctttgagctctggaaggttaatgaaacaactggtgttcaggaaggttccactctggactgtgtcagctttaaaccatcacagaagtcctcaaaccagtataagtaccaattaaaggaactgactgggtgtagggggggtaacacaaggaacacagcctccatctattgtgttcccattctcattagaagacaacccttctggaatcccaccagttattttcatcggtgagattaaatctaatcttgggcaaa

SEQ ID NO: 14 - protein, 267 aa, Bos taurus
RYVSTQGPAHPQPFSSWNDYLGLATLITKAVDGEPRFGCARGGDGGGDGSPPSSSSSSCCSPHVGAGPGALGPALGPPDYDEDDDDDDSDDPGSRSRYLGGALELRALELCADPAEAGLLEERFAELSPFAGRAAAVLLGCAPAAAAAATAEAAPREERAPAWAAEPKLHAASGAAAARLLKPELQVCVFCRNNKEAVALYTTHILKGPDGRVLCPVLRRYTCPLCGASGDNAHTIKYCPLSKVPPPPAARPPPRSARDGLPGKKLR

SEQ ID NO: 15 - DNA, 482 bp, synthetic construct
  misc_feature 1..482: note = Synthetic polynucleotide
  source 1..482: mol_type = other DNA
agttaactaagctttgtacaaaaaagcaggctttaaaggaaccaattcagtcgactggatccggtaccaaggtcgggcaggaagagggcctatttcccatgattccttcatatttgcatatacgatacaaggctgttagagagataattagaattaatttgactgtaaacacaaagatattagtacaaaatacgtgacgtagaaagtaataatttcttgggtagtttgcagttttaaaattatgttttaaaatggactatcatatgcttaccgtaacttgaaagtatttcgatttcttggctttatatatcttgtggaaaggacgaaacaccgaatcgtcgacaagggccaggttttagagctagaaatagcaagttaaaataaggctagtccgttatcaacttgaaaaagtggcaccgagtcggtgctttttttctagacccagctttcttgtacaaagttggcattactcgagatccact

SEQ ID NO: 16 - DNA, 482 bp, synthetic construct; identical to SEQ ID NO: 15
  misc_feature 1..482: note = Synthetic polynucleotide
  source 1..482: mol_type = other DNA

SEQ ID NO: 17 - DNA, 482 bp, synthetic construct
  misc_feature 1..482: note = Synthetic polynucleotide
  source 1..482: mol_type = other DNA
agttaactaagctttgtacaaaaaagcaggctttaaaggaaccaattcagtcgactggatccggtaccaaggtcgggcaggaagagggcctatttcccatgattccttcatatttgcatatacgatacaaggctgttagagagataattagaattaatttgactgtaaacacaaagatattagtacaaaatacgtgacgtagaaagtaataatttcttgggtagtttgcagttttaaaattatgttttaaaatggactatcatatgcttaccgtaacttgaaagtatttcgatttcttggctttatatatcttgtggaaaggacgaaacaccgtggcccttgtcgacgattcgttttagagctagaaatagcaagttaaaataaggctagtccgttatcaacttgaaaaagtggcaccgagtcggtgctttttttctagacccagctttcttgtacaaagttggcattactcgagatccact

SEQ ID NO: 18 - DNA, 318 bp, synthetic construct
  misc_feature 1..318: note = Synthetic polynucleotide
  source 1..318: mol_type = other DNA
tgtacaaaaaagcaggctttaaaggaaccaattcagtcgactggatccggtaccaaggtcgggcaggaagagggcctatttcccatgattccttcatatttgcatatacgatacaaggctgttagagagataattagaattaatttgactgtaaacacaaagatattagtacaaaatacgtgacgtagaaagtaataatttcttgggtagtttgcagttttaaaattatgttttaaaatggactatcatatgcttaccgtaacttgaaagtatttcgatttcttggctttatatatcttgtggaaaggacgaaacacc

SEQ ID NO: 19 - DNA, 20 bp, synthetic construct
  misc_feature 1..20: note = Synthetic oligonucleotide
  source 1..20: mol_type = other DNA
gtggcccttgtcgacgattc

SEQ ID NO: 20 - DNA, 76 bp, synthetic construct
  misc_feature 1..76: note = Synthetic polynucleotide
  source 1..76: mol_type = other DNA
gttttagagctagaaatagcaagttaaaataaggctagtccgttatcaacttgaaaaagtggcaccgagtcggtgc

SEQ ID NO: 21 - skipped

SEQ ID NO: 22 - DNA, 360 bp, synthetic construct
  misc_feature 1..360: note = Synthetic polynucleotide
  source 1..360: mol_type = other DNA
gagggcctatttcccatgattccttcatatttgcatatacgatacaaggctgttagagagataattggaattaatttgactgtaaacacaaagatattagtacaaaatacgtgacgtagaaagtaataatttcttgggtagtttgcagttttaaaattatgttttaaaatggactatcatatgcttaccgtaacttgaaagtatttcgatttcttggctttatatatcttgtggaaaggacgaaacaccgggtcttcgagaagacctgttttagagctagaaatagcaagttaaaataaggctagtccgttatcaacttgaaaaagtggcaccgagtcggtgcttttttgttttagagct

SEQ ID NO: 23 - DNA, 240 bp, synthetic construct
  misc_feature 1..240: note = Synthetic oligonucleotide
  source 1..240: mol_type = other DNA
tttcccatgattccttcatatttgcatatacgatacaaggctgttagagagataattggaattaatttgactgtaaacacaaagatattagtacaaaatacgtgacgtagaaagtaataatttcttgggtagtttgcagttttaaaattatgttttaaaatggactatcatatgcttaccgtaacttgaaagtatttcgatttcttggctttatatatcttgtggaaaggacgaaacacc

SEQ ID NO: 24 - DNA, 76 bp, synthetic construct; identical to SEQ ID NO: 20
  misc_feature 1..76: note = Synthetic oligonucleotide
  source 1..76: mol_type = other DNA

SEQ ID NO: 25 - skipped

SEQ ID NO: 26 - DNA, 61 bp, Sus scrofa
  source 1..61: mol_type = other DNA
cccggtgcccggggcctctggcccttgtcgacgattctggatcagtcccaacaccacctgg

SEQ ID NO: 27 - DNA, 61 bp, Sus scrofa
  source 1..61: mol_type = other DNA
cccggtgcccggggcccttgtcgacgatcagcccttctggatcagtcccaacaccacctgg

SEQ ID NO: 28 - DNA, 356 bp, Sus scrofa
  source 1..356: mol_type = other DNA
tcagcgcttgaccttgcggccggctgaattgcgcccactgcggcgatagagagactgctggccgccgttgagcgggcagtacttgagtgtgtgagcctggtcaccggtggccccgcacaggggacacacatagtgtcgtaggatgggacacaccaccacgccctccggtgtcttcagctggtgcgaggagtacacgtggcgagattccccattgtgtttgcaaaagttgcacagggtggccagccccccgctggccccccgctctcccgggccctggtcctgctccagtgggggctcaggtcttggctcctcaggttgaagtagtccttccacatgtcaaagggtggcagctgcat

SEQ ID NO: 29 - DNA, 56 bp, Sus scrofa
  source 1..56: mol_type = other DNA
ttggctccccggtgcccggggcctctggcccttgtcgacgattctggatcagtccc

SEQ ID NO: 30 - DNA, 56 bp, Sus scrofa; identical to SEQ ID NO: 29
  source 1..56: mol_type = other DNA

SEQ ID NO: 31 - DNA, 49 bp, Sus scrofa
  source 1..49: mol_type = other DNA
ttggctccccggtgcccggggcctctgtcgacgattctggatcagtccc

SEQ ID NO: 32 - DNA, 49 bp, Sus scrofa; identical to SEQ ID NO: 31
  source 1..49: mol_type = other DNA

SEQ ID NO: 33 - DNA, 55 bp, Sus scrofa
  source 1..55: mol_type = other DNA
ttggctcccggtgcccggggcctctggcccttgtcgacgattctggatcagtccc

SEQ ID NO: 34 - DNA, 55 bp, Sus scrofa
  source 1..55: mol_type = other DNA
ttggctccccggtgcccggggcctctgcccttgtccacaattctggatcattccc

SEQ ID NO: 35 - DNA, 49 bp, Sus scrofa; identical to SEQ ID NO: 31
  source 1..49: mol_type = other DNA

SEQ ID NO: 36 - DNA, 55 bp, Sus scrofa
  source 1..55: mol_type = other DNA
ttggctccccggtgcccggtgcccgggcccttgtcgacgattctggatcagtccc

SEQ ID NO: 37 - DNA, 49 bp, Sus scrofa
  source 1..49: mol_type = other DNA
ttggctccccggtgcccggggcccttgtcgacgattctggatcagtccc

SEQ ID NO: 38 - DNA, 54 bp, Sus scrofa
  source 1..54: mol_type = other DNA
ttggctccccggtgcccggggcctctgccttgtcgacgattctggatcagtccc

SEQ ID NO: 39 - DNA, 49 bp, Sus scrofa; identical to SEQ ID NO: 31
  source 1..49: mol_type = other DNA

SEQ ID NO: 40 - DNA, 50 bp, Sus scrofa
  source 1..50: mol_type = other DNA
ttggctccccggtgcccggggccccttgtcgacgattctggatcagtccc

SEQ ID NO: 41 - DNA, 55 bp, Sus scrofa
  source 1..55: mol_type = other DNA
ttggctccccggtgcccggggcctctgcccttgtcgtcaattctggatcagtccc

SEQ ID NO: 42 - DNA, 49 bp, Sus scrofa
  source 1..49: mol_type = other DNA
ttggctccccggtgcccggggcctctgtcgacaattctggatcagtccc

SEQ ID NO: 43 - DNA, 9289 bp, synthetic construct
  misc_feature 1..9289: note = Synthetic polynucleotide
  source 1..9289: mol_type = other DNA
gagggcctatttcccatgattccttcatatttgcatatacgatacaaggctgttagagagataattggaattaatttgactgtaaacacaaagatattagtacaaaatacgtgacgtagaaagtaataatttcttgggtagtttgcagttttaaaattatgttttaaaatggactatcatatgcttaccgtaacttgaaagtatttcgatttcttggctttatatatcttgtggaaaggacgaaacaccgggtcttcgagaagacctgttttagagctagaaatagcaagttaaaataaggctagtccgttatcaacttgaaaaagtggcaccgagtcggtgcttttttgttttagagctagaaatagcaagttaaaataaggctagtccgtttttagcgcgtgcgccaattctgcagacaaatggctctagaggtacccgttacataacttacggtaaatggcccgcctggctgaccgcccaacgacccccgcccattgacgtcaatagtaacgccaatagggactttccattgacgtcaatgggtggagtatttacggtaaactgcccacttggcagtacatcaagtgtatcatatgccaagtacgccccctattgacgtcaatgacggtaaatggcccgcctggcattgtgcccagtacatgaccttatgggactttcctacttggcagtacatctacgtattagtcatcgctattaccatggtcgaggtgagccccacgttctgcttcactctccccatctcccccccctccccacccccaattttgtatttatttattttttaattattttgtgcagcgatgggggcggggggggggggggggcgcgcgccaggcggggcggggcggggcgaggggcggggcggggcgaggcggagaggtgcggcggcagccaatcagagcggcgcgctccgaaagtttccttttatggcgaggcggcggcggcggcggccctataaaaagcgaagcgcgcggcgggcgggagtcgctgcgacgctgccttcgccccgtgccccgctccgccgccgcctcgcgccgcccgccccggctctgactgaccgcgttactcccacaggtgagcgggcgggacggcccttctcctccgggctgtaattagctgagcaagaggtaagggtttaagggatggttggttggtggggtattaatgtttaattacctggagcacctgcctgaaatcaatgacgataagatggccccaaagaagaagcggaaggtcggtatccacggagtcccagcagccgacaagaagtacagcatcggcctggacatcggcaccaactctgtgggctgggccgtgatcaccgacgagtacaaggtgcccagcaagaaattcaaggtgctgggcaacaccgaccggcacagcatcaagaagaacctgatcggagccctgctgttcgacagcggcgaaacagccgaggccacccggctgaagagaaccgccagaagaagatacaccagacggaagaaccggatctgctatctgcaagagatcttcagcaacgagatggccaaggtggacgacagcttcttccacagactggaagagtccttcctggtggaagaggataagaagcacgagcggcaccccatcttcggcaacatcgtggacgaggtggcctaccacgagaagtaccccaccatctaccacctgagaaagaaactggtggacagcaccgacaaggccgacctgcggctgatctatctggccctggcccacatgatcaagttccggggccacttcctgatcgagggcgacctgaaccccgacaacagcgacgtggacaagctgttcatccagctggtgcagacctacaaccagctgttcgaggaaaaccccatcaacgccagcggcgtggacgccaaggccatcctgtctgccagactgagcaagagcagacggctggaaaatctgatcgcccagctgcccggcgagaagaagaatggcctgttcggaaacctgattgccctgagcctgggcctgacccccaacttcaagagcaacttcgacctggccgaggatgccaaactgcagctgagcaaggacacctacgacgacgacctggacaacctgctggcccagatcggcgaccagtacgccgacctgtttctggccgccaagaacctgtccgacgccatcctgctgagcgacatcctgagagtgaacaccgagatcaccaaggcccccctgagcgcctctatgatcaagagatacgacgagcaccaccaggacctgaccctgctgaaagctctcgtgcggcagcagctgcctgagaagtacaaagagattttcttcgaccagagcaagaacggctacgccggctacattgacggcggagccagccaggaagagttctacaagttcatcaagcccatcctggaaaagatggacggcaccgaggaactgctcgtgaagctgaacagagaggacctgctgcggaagcagcggaccttcgacaacggcagcatcccccaccagatccacctgggagagctgcacgccattctgcggcggcaggaagatttttacccattcctgaaggacaaccgggaaaagatcgagaagatcctgaccttccgcatcccctactacgtgggccctctggccaggggaaacagcagattcgcctggatgaccagaaagagcgaggaaaccatcaccccctggaacttcgaggaagtggtggacaagggcgcttccgcccagagcttcatcgagcggatgaccaacttcgataagaacctgcccaacgagaaggtgctgcccaagcacagcctgctgtacgagtacttcaccgtgtataacgagctgaccaaagtgaaatacgtgaccgagggaatgagaaagcccgccttcctgagcggcgagcagaaaaaggccatcgtggacctgctgttcaagaccaaccggaaagtgaccgtgaagcagctgaaagaggactacttcaagaaaatcgagtgcttcgactccgtggaaatctccggcgtggaagatcggttcaacgcctccctgggcacataccacgatctgctgaaaattatcaaggacaaggacttcctggacaatgaggaaaacgaggacattctggaagatatcgtgctgaccctgacactgtttgaggacagagagatgatcgaggaacggctgaaaacctatgcccacctgttcgacgacaaagtgatgaagcagctgaagcggcggagatacaccggctggggcaggctgagccggaagctgatcaacggcatccgggacaagcagtccggcaagacaatcctggatttcctgaagtccgacggcttcgccaacagaaacttcatgcagctgatccacgacgacagcctgacctttaaagaggacatccagaaagcccaggtgtccggccagggcgatagcctgcacgagcacattgccaatctggccggcagccccgccattaagaagggcatcctgcagacagtgaaggtggtggacgagctcgtgaaagtgatgggccggcacaagcccgagaacatcgtgatcgaaatggccagagagaaccagaccacccagaagggacagaagaacagccgcgagagaatgaagcggatcgaagagggcatcaaagagctgggcagccagatcctgaaagaacaccccgtggaaaacacccagctgcagaacgagaagctgtacctgtactacctgcagaatgggcgggatatgtacgtggaccaggaactggacatcaaccggctgtccgactacgatgtggaccatatcgtgcctcagagctttctgaaggacgactccatcgacaacaaggtgctgaccagaagcgacaagaaccggggcaagagcgacaacgtgccctccgaagaggtcgtgaagaagatgaagaactactggcggcagctgctgaacgccaagctgattacccagagaaagttcgacaatctgaccaaggccgagagaggcggcctgagcgaactggataaggccggcttcatcaagagacagctggtggaaacccggcagatcacaaagcacgtggcacagatcctggactcccggatgaacactaagtacgacgagaatgacaagctgatccgggaagtgaaagtgatcaccctgaagtccaagctggtgtccgatttccggaaggatttccagttttacaaagtgcgcgagatcaacaactaccaccacgcccacgacgcctacctgaacgccgtcgtgggaaccgccctgatcaaaaagtaccctaagctggaaagcgagttcgtgtacggcgactacaaggtgtacgacgtgcggaagatgatcgccaagagcgagcaggaaatcggcaaggctaccgccaagtacttcttctacagcaacatcatgaactttttcaagaccgagattaccctggccaacggcgagatccggaagcggcctctgatcgagacaaacggcgaaaccggggagatcgtgtgggataagggccgggattttgccaccgtgcggaaagtgctgagcatgccccaagtgaatatcgtgaaaaagaccgaggtgcagacaggcggcttcagcaaagagtctatcctgcccaagaggaacagcgataagctgatcgccagaaagaaggactgggaccctaagaagtacggcggcttcgacagccccaccgtggcctattctgtgctggtggtggccaaagtggaaaagggcaagtccaagaaactgaagagtgtgaaagagctgctggggatcaccatcatggaaagaagcagcttcgagaagaatcccatcgactttctggaagccaagggctacaaagaagtgaaaaaggacctgatcatcaagctgcctaagtactccctgttcgagctggaactttttttcaggttggaccggtgccaccatggactataaggaccacgacggagactacaaggatcatgatattgattacaaagacgaacggccggaagagaatgctggcctctgccggcgaactgcagaagggaaacgaactggccctgccctccaaatatgtgaacttcctgtacctggccagccactatgagaagctgaagggctcccccgaggataatgagcagaaacagctgtttgtggaacagcacaagcactacctggacgagatcatcgagcagatcagcgagttctccaagagagtgatcctggccgacgctaatctggacaaagtgctgtccgcctacaacaagcaccgggataagcccatcagagagcaggccgagaatatcatccacctgtttaccctgaccaatctgggagcccctgccgccttcaagtactttgacaccaccatcgaccggaagaggtacaccagcaccaaagaggtgctggacgccaccctgatccaccagagcatcaccggcctgtacgagacacggatcgacctgtctcagctgggaggcgacaaaaggccggcggccacgaaaaaggccggccaggcaaaaaagaaaaaggaattcggcagtggagagggcagaggaagtctgctaacatgcggtgacgtcgaggagaatcctggcccagtgagcaagggcgaggagctgttcaccggggtggtgcccatcctggtcgagctggacggcgacgtaaacggccacaagttcagcgtgtccggcgagggcgagggcgatgccacctacggcaagctgaccctgaagttcatctgcaccaccggcaagctgcccgtgccctggcccaccctcgtgaccaccctgacctacggcgtgcagtgcttcagccgctaccccgaccacatgaagcagcacgacttcttcaagtccgccatgcccgaaggctacgtccaggagcgcaccatcttcttcaaggacgacggcaactacaagacccgcgccgaggtgaagttcgagggcgacaccctggtgaaccgcatcgagctgaagggcatcgacttcaaggaggacggcaacatcctggggcacaagctggagtacaactacaacagccacaacgtctatatcatggccgacaagcagaagaacggcatcaaggtgaacttcaagatccgccacaacatcgaggacggcagcgtgcagctcgccgaccactaccagcagaacacccccatcggcgacggccccgtgctgctgcccgacaaccactacctgagcacccagtccgccctgagcaaagaccccaacgagaagcgcgatcacatggtcctgctggagttcgtgaccgccgccgggatcactctcggcatggacgagctgtacaaggaattctaactagagctcgctgatcagcctcgactgtgccttctagttgccagccatctgttgtttgcccctcccccgtgccttccttgaccctggaaggtgccactcccactgtcctttcctaataaaatgaggaaattgcatcgcattgtctgagtaggtgtcattctattctggggggtggggtggggcaggacagcaagggggaggattgggaagagaatagcaggcatgctggggagcggccgcaggaacccctagtgatggagttggccactccctctctgcgcgctcgctcgctcactgaggccgggcgaccaaaggtcgcccgacgcccgggctttgcccgggcggcctcagtgagcgagcgagcgcgcagctgcctgcaggggcgcctgatgcggtattttctccttacgcatctgtgcggtatttcacaccgcatacgtcaaagcaaccatagtacgcgccctgtagcggcgcattaagcgcggcgggtgtggtggttacgcgcagcgtgaccgctacacttgccagcgccctagcgcccgctcctttcgctttcttcccttcctttctcgccacgttcgccggctttccccgtcaagctctaaatcgggggctccctttagggttccgatttagtgctttacggcacctcgaccccaaaaaacttgatttgggtgatggttcacgtagtgggccatcgccctgatagacggtttttcgccctttgacgttggagtccacgttctttaatagtggactcttgttccaaactggaacaacactcaaccctatctcgggctattcttttgatttataagggattttgccgatttcggcctattggttaaaaaatgagctgatttaacaaaaatttaacgcgaattttaacaaaatattaacgtttacaattttatggtgcactctcagtacaatctgctctgatgccgcatagttaagccagccccgacacccgccaacacccgctgacgcgccctgacgggcttgtctgctcccggcatccgcttacagacaagctgtgaccgtctccgggagctgcatgtgtcagaggttttcaccgtcatcaccgaaacgcgcgagacgaaagggcctcgtgatacgcctatttttataggttaatgtcatgataataatggtttcttagacgtcaggtggcacttttcggggaaatgtgcgcggaacccctatttgtttatttttctaaatacattcaaatatgtatccgctcatgagacaataaccctgataaatgcttcaataatattgaaaaaggaagagtatgagtattcaacatttccgtgtcgcccttattcccttttttgcggcattttgccttcctgtttttgctcacccagaaacgctggtgaaagtaaaagatgctgaagatcagttgggtgcacgagtgggttacatcgaactggatctcaacagcggtaagatccttgagagttttcgccccgaagaacgttttccaatgatgagcacttttaaagttctgctatgtggcgcggtattatcccgtattgacgccgggcaagagcaactcggtcgccgcatacactattctcagaatgacttggttgagtactcaccagtcacagaaaagcatcttacggatggcatgacagtaagagaattatgcagtgctgccataaccatgagtgataacactgcggccaacttacttctgacaacgatcggaggaccgaaggagctaaccgcttttttgcacaacatgggggatcatgtaactcgccttgatcgttgggaaccggagctgaatgaagccataccaaacgacgagcgtgacaccacgatgcctgtagcaatggcaacaacgttgcgcaaactattaactggcgaactacttactctagcttcccggcaacaattaatagactggatggaggcggataaagttgcaggaccacttctgcgctcggcccttccggctggctggtttattgctgataaatctggagccggtgagcgtggaagccgcggtatcattgcagcactggggccagatggtaagccctcccgtatcgtagttatctacacgacggggagtcaggcaactatggatgaacgaaatagacagatcgctgagataggtgcctcactgattaagcattggtaactgtcagaccaagtttactcatatatactttagattgatttaaaacttcatttttaatttaaaaggatctaggtgaagatcctttttgataatctcatgaccaaaatcccttaacgtgagttttcgttccactgagcgtcagaccccgtagaaaagatcaaaggatcttcttgagatcctttttttctgcgcgtaatctgctgcttgcaaacaaaaaaaccaccgctaccagcggtggtttgtttgccggatcaagagctaccaactctttttccgaaggtaactggcttcagcagagcgcagataccaaatactgtccttctagtgtagccgtagttaggccaccacttcaagaactctgtagcaccgcctacatacctcgctctgctaatcctgttaccagtggctgctgccagtggcgataagtcgtgtcttaccgggttggactcaagacgatagttaccggataaggcgcagcggtcgggctgaacggggggttcgtgcacacagcccagcttggagcgaacgacctacaccgaactgagatacctacagcgtgagctatgagaaagcgccacgcttcccgaagggagaaaggcggacaggtatccggtaagcggcagggtcggaacaggagagcgcacgagggagcttccagggggaaacgcctggtatctttatagtcctgtcgggtttcgccacctctgacttgagcgtcgatttttgtgatgctcgtcaggggggcggagcctatggaaaaacgccagcaacgcggcctttttacggttcctggccttttgctggccttttgctcacatgt

SEQ ID NO: 44 - DNA, 61 bp, Sus scrofa
  source 1..61: mol_type = other DNA
ctcaggtcttggctccccggtgcccggggcctctggcccttgtcgacgattctggatcagt

SEQ ID NO: 45 - DNA, 60 bp, Sus scrofa
  source 1..60: mol_type = other DNA
ctcaggtcttggctccccggtgcccggggcctctgcccttgtcgacgattctggatcagt

SEQ ID NO: 46 - DNA, 60 bp, Sus scrofa
  source 1..60: mol_type = other DNA
ctcaggtcttggctccccggtgcccggtgcccgggcccttgtcgacgattctggatcagt

SEQ ID NO: 47 - DNA, 60 bp, Sus scrofa; identical to SEQ ID NO: 46
  source 1..60: mol_type = other DNA

SEQ ID NO: 48 - DNA, 54 bp, Sus scrofa
  misc_feature 6..7: note = n is a, c, g, or t
  source 1..54: mol_type = other DNA
atcagnncttggctccccggtgcccggggcctctggccacgattctggatcagt

SEQ ID NO: 49 - DNA, 54 bp, Sus scrofa
  source 1..54: mol_type = other DNA
ctcaggtcttggctccccggtgcccggggcctctgtcgacgattctggatcagt

SEQ ID NO: 50 - DNA, 54 bp, Sus scrofa; identical to SEQ ID NO: 49
  source 1..54: mol_type = other DNA

SEQ ID NO: 51 - DNA, 59 bp, Sus scrofa
  source 1..59: mol_type = other DNA
ctcaggtcttggctccccggtgcccggggcctctggcccttgtcgacttctggatcagt

SEQ ID NO: 52 - DNA, 60 bp, Sus scrofa; identical to SEQ ID NO: 45
  source 1..60: mol_type = other DNA

SEQ ID NO: 53 - DNA, 24 bp, Sus scrofa
  source 1..24: mol_type = other DNA
gcaccagctgaagaccaccggagg

SEQ ID NO: 54 - DNA, 23 bp, Sus scrofa
  source 1..23: mol_type = other DNA
gctggtgcgaggagtacacgtgg

SEQ ID NO: 55 - DNA, 65 bp, Sus scrofa
  source 1..65: mol_type = other DNA
gaatctcgccacgtgtactcctcgcaccagctgaagacaccggagggcgtggtggtgtgtcccat

SEQ ID NO: 56 - DNA, 64 bp, Sus scrofa
  source 1..64: mol_type = other DNA
gaatctcgccacgtgtactcctcgcaccagctgaagacaccggagggcgtggtggtgttcccat

SEQ ID NO: 57 - DNA, 65 bp, Sus scrofa; identical to SEQ ID NO: 55
  source 1..65: mol_type = other DNA

SEQ ID NO: 58 - DNA, 64 bp, Sus scrofa; identical to SEQ ID NO: 56
  source 1..64: mol_type = other DNA

SEQ ID NO: 59 - DNA, 65 bp, Sus scrofa; identical to SEQ ID NO: 55
  source 1..65: mol_type = other DNA

SEQ ID NO: 60 - DNA, 65 bp, Sus scrofa; identical to SEQ ID NO: 55
  source 1..65: mol_type = other DNA

SEQ ID NO: 61 - DNA, 65 bp, Sus scrofa; identical to SEQ ID NO: 55
  source 1..65: mol_type = other DNA

SEQ ID NO: 62 - DNA, 1000 bp, Bos taurus
  source 1..1000: mol_type = other DNA
gaaggatgggggtgggggcgtttgcagacatgaagttttgttgaaaggacagaaaaactgaggcccagggagacgggtctttccagaggtcacagagcaccttgcaggccaagcaagcaccagagacaacaggaaagacccccttccacatctccatggggaattaaagtcagaaggaatcaaaggtgaggagtgggccctttaaatcctaagctccacctttgcttagaagggtctttgggaatataaaagggggtgcagttcctctctgctcctgaaaaccatcagctgctcctgtctgcgggcccccagcccacttctctccagccacccaccaccaacactcccccgggtgccatgcagctgccaccctttgacatgtggaaggactacttcaacctgagccaagtggtgctggcactgatccagagtcgggggcaagggttggagacccaagggactggggagccgagacccgggccccatgtggagcaggatcaggggcagggcggacgcggggctggcgggggcctggccaccctgtgcaacttttgcaaacacaatggagagtctcgccacgtgtactcctcacaccagctgaagaccccggagggcgtggtggtgtgtcccattctgcggcattatgtatgtcccctgtgcggggccaccggggaccaggcccacacactcaagtactgcccactcaacggaggacagcagtctctctaccgccgcagtgggcgcaactcagccggccgcaaggtcaagcgctgaagaccgtcaggtacccacccgctgcagccccaaccctccctggttcagccctcccaagcccctggactctccccatctatggactcgtcaggccctttggaatgtctgactctcagtacttgatccctgctggatcctggaacaacggaggcagtgggaagccaggccaactccgcggccccttagaactctcagctctccggactcttgtctgcgagtgtctgtg

SEQ ID NO: 63 - DNA, 417 bp, Bos taurus
  source 1..417: mol_type = other DNA
atgcagctgccaccctttgacatgtggaaggactacttcaacctgagccaagtggtgctggcactgatccagagtcgggggcaagggttggagacccaagggactggggagccgagacccgggccccatgtggagcaggatcaggggcagggcggacgcggggctggcgggggcctggccaccctgtgcaacttttgcaaacacaatggagagtctcgccacgtgtactcctcacaccagctgaagaccccggagggcgtggtggtgtgtcccattctgcggcattatgtatgtcccctgtgcggggccaccggggaccaggcccacacactcaagtactgcccactcaacggaggacagcagtctctctaccgccgcagtgggcgcaactcagccggccgcaaggtcaagcgctga

SEQ ID NO: 64 - DNA, 20 bp, synthetic construct
  misc_feature 1..20: note = primer
  source 1..20: mol_type = other DNA
agacgggtctttccagaggt

SEQ ID NO: 65 - DNA, 20 bp, Bos taurus
  source 1..20: mol_type = other DNA
aagctccacctttgcttaga

SEQ ID NO: 66 - DNA, 21 bp, Bos taurus
  source 1..21: mol_type = other DNA
ctttgcttagaagggtctttt

SEQ ID NO: 67 - DNA, 20 bp, Bos taurus
  source 1..20: mol_type = other DNA
ggtctttgggaatataaaag

SEQ ID NO: 68 - DNA, 19 bp, Bos taurus
  source 1..19: mol_type = other DNA
ggcaagggttggagaccca

SEQ ID NO: 69 - DNA, 20 bp, Bos taurus
  source 1..20: mol_type = other DNA
gccgagacccgggccccatg

SEQ ID NO: 70 - DNA, 20 bp, Bos taurus
  source 1..20: mol_type = other DNA
cccatgtggagcaggatcag

SEQ ID NO: 71 - DNA, 19 bp, Bos taurus
  source 1..19: mol_type = other DNA
tccccatctctggactcgt

SEQ ID NO: 72 - DNA, 20 bp, Bos taurus
  source 1..20: mol_type = other DNA
tctggactcgtccggccctt

SEQ ID NO: 73 - DNA, 20 bp, Bos taurus
  source 1..20: mol_type = other DNA
tctcagtacttgatccctgc

SEQ ID NO: 74 - DNA, 20 bp, synthetic construct
  misc_feature 1..20: note = primer
  source 1..20: mol_type = other DNA
acaagagtccggagagctga

SEQ ID NO: 75 - DNA, 54 bp, Sus scrofa
  source 1..54: mol_type = other DNA
tgccatgcagctgccaccctttgacatgtggaaggactacttcaacctgagcca

SEQ ID NO: 76 - DNA, 18 bp, Sus scrofa
  source 1..18: mol_type = other DNA
tgccatgcagctgccacc

SEQ ID NO: 77 - DNA, 18 bp, Sus scrofa
  source 1..18: mol_type = other DNA
tggctcaggttgaagtag

SEQ ID NO: 78 - DNA, 52 bp, Sus scrofa
  source 1..52: mol_type = other DNA
tttgacatgtggaaggactacttcaacctgagccaggtggtgttgggactga

SEQ ID NO: 79 - DNA, 18 bp, Sus scrofa
  source 1..18: mol_type = other DNA
tttgacatgtggaaggac

SEQ ID NO: 80 - DNA, 18 bp, Sus scrofa
  source 1..18: mol_type = other DNA
tcagtcccaacaccacct

SEQ ID NO: 81 - DNA, 53 bp, Sus scrofa
  source 1..53: mol_type = other DNA
tcaacctgagccaggtggtgttgggactgatccagaatcgtcgacaagggcca

SEQ ID NO: 82 - DNA, 18 bp, Sus scrofa
  source 1..18: mol_type = other DNA
tcaacctgagccaggtgg

SEQ ID NO: 83 - DNA, 18 bp, Sus scrofa
  source 1..18: mol_type = other DNA
tggcccttgtcgacgatt

SEQ ID NO: 84 - DNA, 20 bp, Sus scrofa
  source 1..20: mol_type = other DNA
agcgggcagtacttgagtgt

SEQ ID NO: 85 - DNA, 20 bp, Sus scrofa
  source 1..20: mol_type = other DNA
ccagaaaaccttctgctgct

SEQ ID NO: 86 - DNA, 26 bp, Sus scrofa
  source 1..26: mol_type = other DNA
ccagaatcgtcgacaagggccagagg

SEQ ID NO: 87 - DNA, 26 bp, Sus scrofa
  source 1..26: mol_type = other DNA
ggtcttagcagctgttcccggtctcc

SEQ ID NO: 88 - DNA, 24 bp, synthetic construct
  misc_feature 1..24: note = forward oligo for bovine NANOS2
  source 1..24: mol_type = other DNA
caccggtctttgggaatataaaag

SEQ ID NO: 89 - DNA, 24 bp, synthetic construct
  misc_feature 1..24: note = reverse oligo for bovine NANOS2
  source 1..24: mol_type = other DNA
aaaccttttatattcccaaagacc

SEQ ID NO: 90 - DNA, 23 bp, synthetic construct
  misc_feature 1..23: note = forward oligo for bovine NANOS2
  source 1..23: mol_type = other DNA
caccgtctttgggaatataaaag

SEQ ID NO: 91 - DNA, 23 bp, synthetic construct
  misc_feature 1..23: note = reverse oligo for bovine NANOS2
  source 1..23: mol_type = other DNA
aaaccttttatattcccaaagac

SEQ ID NO: 92 - DNA, 25 bp, synthetic construct
  misc_feature 1..25: note = forward oligo for bovine NANOS2
  source 1..25: mol_type = other DNA
caccgctttgcttagaagggtcttt

SEQ ID NO: 93 - DNA, 25 bp, synthetic construct
  misc_feature 1..25: note = reverse oligo for bovine NANOS2
  source 1..25: mol_type = other DNA
aaacaaagacccttctaagcaaagc

SEQ ID NO: 94 - DNA, 23 bp, synthetic construct
  misc_feature 1..23: note = forward oligo for bovine NANOS2
  source 1..23: mol_type = other DNA
caccgttgcttagaagggtcttt

SEQ ID NO: 95 - DNA, 23 bp, synthetic construct
  misc_feature 1..23: note = reverse oligo for bovine NANOS2
  source 1..23: mol_type = other DNA
aaacaaagacccttctaagcaac

SEQ ID NO: 96 - DNA, 25 bp, synthetic construct
  misc_feature 1..25: note = forward oligo for bovine NANOS2
  source 1..25: mol_type = other DNA
caccgagctccacctttgcttagaa

SEQ ID NO: 97 - DNA, 25 bp, synthetic construct
  misc_feature 1..25: note = reverse oligo for bovine NANOS2
  source 1..25: mol_type = other DNA
aaacttctaagcaaaggtggagctc

SEQ ID NO: 98 - DNA, 23 bp, synthetic construct
  misc_feature 1..23: note = forward oligo for bovine NANOS2
  source 1..23: mol_type = other DNA
caccgctccacctttgcttagaa

SEQ ID NO: 99 - DNA, 23 bp, synthetic construct
  misc_feature 1..23: note = reverse oligo for bovine NANOS2
  source 1..23: mol_type = other DNA
aaacttctaagcaaaggtggagc

SEQ ID NO: 100 - DNA, 24 bp, synthetic construct
  misc_feature 1..24: note = forward oligo for bovine NANOS2
  source 1..24: mol_type = other DNA
caccggcaagggttggagacccaa

SEQ ID NO: 101 - DNA, 24 bp, synthetic construct
  misc_feature 1..24: note = reverse oligo for bovine NANOS2
  source 1..24: mol_type = other DNA
aaacttgggtctccaacccttgcc

SEQ ID NO: 102 - DNA, 23 bp, synthetic construct
  misc_feature 1..23: note = forward oligo for bovine NANOS2
  source 1..23: mol_type = other DNA
caccgcaagggttggagacccaa

SEQ ID NO: 103 - DNA, 23 bp, synthetic construct
  misc_feature 1..23: note = reverse oligo for bovine NANOS2
  source 1..23: mol_type = other DNA
aaacttgggtctccaacccttgc

SEQ ID NO: 104 - DNA, 24 bp, synthetic construct
  misc_feature 1..24: note = forward oligo for bovine NANOS2
  source 1..24: mol_type = other DNA
caccgccgagacccgggccccatg

SEQ ID NO: 105 - DNA, 24 bp, synthetic construct
  misc_feature 1..24: note = reverse oligo for bovine NANOS2
  source 1..24: mol_type = other DNA
aaaccatggggcccgggtctcggc

SEQ ID NO: 106 - DNA, 21 bp, synthetic construct
  misc_feature 1..21: note = forward oligo for bovine NANOS2
  source 1..21: mol_type = other DNA
caccgagacccgggccccatg

SEQ ID NO: 107 - DNA, 21 bp, synthetic construct
  misc_feature 1..21: note = reverse oligo for bovine NANOS2
  source 1..21: mol_type = other DNA
aaaccatggggcccgggtctc

SEQ ID NO: 108 - DNA, 25 bp, synthetic construct
  misc_feature 1..25: note = forward oligo for bovine NANOS2
  source 1..25: mol_type = other DNA
caccgcccatgtggagcaggatcag

SEQ ID NO: 109 - DNA, 25 bp, synthetic construct
  misc_feature 1..25: note = reverse oligo for bovine NANOS2
  source 1..25: mol_type = other DNA
aaacctgatcctgctccacatgggc

SEQ ID NO: 110 - DNA, 23 bp, synthetic construct
  misc_feature 1..23: note = forward oligo for bovine NANOS2
  source 1..23: mol_type = other DNA
caccgcatgtggagcaggatcag

SEQ ID NO: 111 - DNA, 23 bp, synthetic construct
  misc_feature 1..23: note = reverse oligo for bovine NANOS2
  source 1..23: mol_type = other DNA
aaacctgatcctgctccacatgc

SEQ ID NO: 112 - DNA, 25 bp, synthetic construct
  misc_feature 1..25: note = forward oligo for bovine NANOS2
  source 1..25: mol_type = other DNA
caccgtccccatctctggactcgtc

SEQ ID NO: 113 - DNA, 25 bp, synthetic construct
  misc_feature 1..25: note = reverse oligo for bovine NANOS2
  source 1..25: mol_type = other DNA
aaacgacgagtccagagatggggac

SEQ ID NO: 114 - DNA, 23 bp, synthetic construct
  misc_feature 1..23: note = forward oligo for bovine NANOS2
  source 1..23: mol_type = other DNA
caccgcccatctctggactcgtc

SEQ ID NO: 115 - DNA, 23 bp, synthetic construct
  misc_feature 1..23: note = reverse oligo for bovine NANOS2
  source 1..23: mol_type = other DNA
aaacgacgagtccagagatgggc

SEQ ID NO: 116 - DNA, 25 bp, synthetic construct
  misc_feature 1..25: note = forward oligo for bovine NANOS2
  source 1..25: mol_type = other DNA
caccgtctggactcgtccggccctt

SEQ ID NO: 117 - DNA, 201 bp, Bos taurus
  source 1..201: mol_type = other DNA
tgggccctttaaatcctaagctccacctttgcttagaagggtctttgggaatataaaagggggtgcagttcctgagccaagtggtgctggcactgatccagagtcgggggcaagggttggagacccaagggactggggagccgagacccggccccatgtggagcaggatcaggggcagggcggacgcggggccggcggggg

SEQ ID NO: 118 - DNA, 132 bp, Bos taurus
  source 1..132: mol_type = other DNA
tgggccctttaaatcctaagctccacctttgcttagaagggtctttgggaatataacaagggactggggagccgagacccggccccatgtggagcaggatcaggggcagggcggacgcggggccggcggggg

SEQ ID NO: 119 - DNA, 132 bp, Bos taurus; identical to SEQ ID NO: 118
  source 1..132: mol_type = other DNA

SEQ ID NO: 120 - DNA, 119 bp, Bos taurus
  source 1..119: mol_type = other DNA
tgggccctttaaatcctaagctccacctttgcttagaagggtctttgggactggggagccgagacccggccccatgtggagcaggatcaggggcagggcggacgcggggccggcggggg

SEQ ID NO: 121 - DNA, 119 bp, Bos taurus; identical to SEQ ID NO: 120
  source 1..119: mol_type = other DNA

SEQ ID NO: 122 - DNA, 112 bp, Bos taurus
  source 1..112: mol_type = other DNA
tgggccctttaaatcctaagctccacctttgcttagaagggtctttgggagccgagacccggccccatgtggagcaggatcaggggcagggcggacgcggggccggcggggg

SEQ ID NO: 123 - DNA, 201 bp, Bos taurus; identical to SEQ ID NO: 117
  source 1..201: mol_type = other DNA

SEQ ID NO: 124 - DNA, 129 bp, Bos taurus
  source 1..129: mol_type = other DNA
tgggccctttaaatcctaagctccacctttgcttagaagggtctttgggggtgcagttcctgagccaagtggtgctggcactgatccagagtcgggggcaagggttggagacccaagggactggggagc

SEQ ID NO: 125 - DNA, 103 bp, Bos taurus
  source 1..103: mol_type = other DNA
tgggccctttaaatcctaagctccacctttgcttagaagggtctttgggaatataacatgtggagcaggatcaggggcagggcggacgcggggccggcggggg

SEQ ID NO: 126 - DNA, 104 bp, Bos taurus
  source 1..104: mol_type = other DNA
tgggccctttaaatcctaagctccacctttgcttagaagggtctttgggaatataaacatgtggagcaggatcaggggcagggcggacgcggggccggcggggg

SEQ ID NO: 127 - DNA, 106 bp, Bos taurus
  source 1..106: mol_type = other DNA
tgggccctttaaatcctaagctccacctttgcttagaagggtctttgggagtgcagttccatgtggagcaggatcaggggcagggcggacgcggggccggcggggg

SEQ ID NO: 128 - DNA, 103 bp, Bos taurus; identical to SEQ ID NO: 125
  source 1..103: mol_type = other DNA

SEQ ID NO: 129 - DNA, 201 bp, Bos taurus; identical to SEQ ID NO: 117
  source 1..201: mol_type = other DNA

SEQ ID NO: 130 - DNA, 48 bp, Bos taurus
  source 1..48: mol_type = other DNA
tgggccctttaaatcctaagctccacctttgcttagaagggtctaagg

SEQ ID NO: 131 - DNA, 89 bp, Bos taurus
  source 1..89: mol_type = other DNA
tgggccctttaaatcctaagctccacctttgcttagaagggtctttgggaatataatcaggggcagggcggacgcggggccggcggggg

SEQ ID NO: 132 - DNA, 88 bp, Bos taurus
  source 1..88: mol_type = other DNA
tgggccctttaaatcctaagctccacctttgcttagaagggtctttgggaatataacaggggcagggcggacgcggggccggcggggg

SEQ ID NO: 133 - DNA, 45 bp, Bos taurus
  source 1..45: mol_type = other DNA
tgggccctttaaatcctaagctccacctttgctggccgggggggg

SEQ ID NO: 134 - DNA, 62 bp, Bos taurus
  source 1..62: mol_type = other DNA
tgggccctttaaatcctaagctccacctttgcttagaagggcggacgcggggccggcggggg

SEQ ID NO: 135 - DNA, 200 bp, Bos taurus
  source 1..200: mol_type = other DNA
tgggccctttaaatcctaagctccacctttgcttagaagggtctttgggaatataaaagggggtgcagttcctgagccaagtggtgctggcactgatccagagtcgggggcaagggttggagacccaagggactggggagccgagacccggccccatgtggagcaggatcaggggcagggcggacgcggggccggcgggg

SEQ ID NO: 136 - DNA, 132 bp, Bos taurus; identical to SEQ ID NO: 118
  source 1..132: mol_type = other DNA

SEQ ID NO: 137 - DNA, 132 bp, Bos taurus; identical to SEQ ID NO: 118
  source 1..132: mol_type = other DNA

SEQ ID NO: 138 - DNA, 132 bp, Bos taurus; identical to SEQ ID NO: 118
  source 1..132: mol_type = other DNA

SEQ ID NO: 139 - DNA, 132 bp, Bos taurus; identical to SEQ ID NO: 118
  source 1..132: mol_type = other DNA

SEQ ID NO: 140 - DNA, 132 bp, Bos taurus; identical to SEQ ID NO: 118
  source 1..132: mol_type = other DNA

SEQ ID NO: 141 - DNA, 201 bp, Bos taurus; identical to SEQ ID NO: 117
  source 1..201: mol_type = other DNA

SEQ ID NO: 142 - DNA, 98 bp, Bos taurus
  source 1..98: mol_type = other DNA
tgggccctttaaatcctaagctccacctttgcttagaagggtctttgggaatatgtggagcaggatcaggggcagggcggacgcggggccggcggggg

SEQ ID NO: 143 - DNA, 103 bp, Bos taurus; identical to SEQ ID NO: 125
  source 1..103: mol_type = other DNA

SEQ ID NO: 144 - DNA, 89 bp, Bos taurus
  source 1..89: mol_type = other DNA
tgggccctttaaatcctaagctccacctttgcttagaagggtctttgggaatatgatcaggggcagggcggacgcggggccggcggggg

SEQ ID NO: 145 - DNA, 89 bp, Bos taurus
  source 1..89: mol_type = other DNA
tgggccctttaaatcctaagctccacctttgcttagaagggtctttgggagcaggatcaggggcagggcggacgcggggccggcggggg

SEQ ID NO: 146 - DNA, 103 bp, Bos taurus; identical to SEQ ID NO: 125
  source 1..103: mol_type = other DNA

SEQ ID NO: 147 - DNA, 201 bp, Bos taurus; identical to SEQ ID NO: 117
  source 1..201: mol_type = other DNA

SEQ ID NO: 148 - DNA, 68 bp, Bos taurus
  source 1..68: mol_type = other DNA
tgggccctttaaatcctaagctccacctttgcttctcaggggcagggcggacgcggggccggcggggg

SEQ ID NO: 149 - DNA, 70 bp, Bos taurus
  source 1..70: mol_type = other DNA
tgggccctttaaatcctaagctccacctttgcttagaagggtctttgggcggacgcggggccggcggggg

SEQ ID NO: 150 - DNA, 88 bp, Bos taurus
  source 1..88: mol_type = other DNA
gggccctttaaatcctaagctccacctttgcttagaagggtctttgggaatataatcaggggcagggcggacgcggggccggcggggg

SEQ ID NO: 151 - DNA, 67 bp, Bos taurus
  source 1..67: mol_type = other DNA
tgggccctttaaatcctaagctccacctttgcttagaagggcagggcggacgcggggccggcggggg

SEQ ID NO: 152 - DNA, 125 bp, Bos taurus
  source 1..125: mol_type = other DNA
tgggccctttaaatcctaagctccacctttgcttagaagtggtgctggcactgatccagagtcgggggcaagggttggagacccaagggactggggagccgagacccggccccatgtggagcagg

SEQ ID NO: 153 - DNA, 25 bp, synthetic construct
  misc_feature 1..25: note = reverse oligo for bovine NANOS2
  source 1..25: mol_type = other DNA
aaacaagggccggacgagtccagac

SEQ ID NO: 154 - DNA, 21 bp, synthetic construct
  misc_feature 1..21: note = forward oligo for bovine NANOS2
  source 1..21: mol_type = other DNA
caccggactcgtccggccctt

SEQ ID NO: 155 - DNA, 21 bp, synthetic construct
  misc_feature 1..21: note = reverse oligo for bovine NANOS2
  source 1..21: mol_type = other DNA
aaacaagggccggacgagtcc

SEQ ID NO: 156 - DNA, 25 bp, synthetic construct
  misc_feature 1..25: note = forward oligo for bovine NANOS2
  source 1..25: mol_type = other DNA
caccgtctcagtacttgatccctgc

SEQ ID NO: 157 - DNA, 25 bp, synthetic construct
  misc_feature 1..25: note = reverse oligo for bovine NANOS2
  source 1..25: mol_type = other DNA
aaacgcagggatcaagtactgagac

SEQ ID NO: 158 - DNA, 23 bp, synthetic construct
  misc_feature 1..23: note = forward oligo for bovine NANOS2
  source 1..23: mol_type = other DNA
caccgtcagtacttgatccctgc

SEQ ID NO: 159 - DNA, 23 bp, synthetic construct
  misc_feature 1..23: note = reverse oligo for bovine NANOS2
  source 1..23: mol_type = other DNA
aaacgcagggatcaagtactgac

SEQ ID NO: 160 - DNA, 22 bp, Sus scrofa
  source 1..22: mol_type = other DNA
gatcagtcccaacaccacctgg

SEQ ID NO: 161 - DNA, 22 bp, Sus scrofa
  source 1..22: mol_type = other DNA
ccaggtggtgttgggactgatc

SEQ ID NO: 162 - DNA, 23 bp, Sus scrofa
  source 1..23: mol_type = other DNA
gaatcgtcgacaagggccagagg

SEQ ID NO: 163 - DNA, 42 bp, Sus scrofa
  source 1..42: mol_type = other DNA
ctacttcaacctgagccaggtggtgttgggactgatccagaa

SEQ ID NO: 164 - DNA, 37 bp, Sus scrofa
  source 1..37: mol_type = other DNA
ctacttcaacctgagccaggttgggactgatccagaa

SEQ ID NO: 165 - DNA, 39 bp, Sus scrofa
  source 1..39: mol_type = other DNA
ctacttcaacctgagccaggtgttgggactgatccagaa

SEQ ID NO: 166 - DNA, 39 bp, Sus scrofa
  source 1..39: mol_type = other DNA
ctacttcaacctgagccagggactgggactgatccagaa

SEQ ID NO: 167 - DNA, 43 bp, Sus scrofa
  source 1..43: mol_type = other DNA
ctacttcaacctgagccaggtgggtgttgggactgatccagaa

SEQ ID NO: 168 - DNA, 41 bp, Sus scrofa
  source 1..41: mol_type = other DNA
ctacttcaacctgagccaggtgtgttgggactgatccagaa

SEQ ID NO: 169 - DNA, 37 bp, Sus scrofa
  source 1..37: mol_type = other DNA
ctacttcaacctgagccaggttgggaccgatccagaa

SEQ ID NO: 170 - DNA, 39 bp, Sus scrofa; identical to SEQ ID NO: 165
  source 1..39: mol_type = other DNA

SEQ ID NO: 171 - DNA, 39 bp, Sus scrofa; identical to SEQ ID NO: 165
  source 1..39: mol_type = other DNA

SEQ ID NO: 172 - DNA, 32 bp, Sus scrofa
  source 1..32: mol_type = other DNA
ctacttcaacctgagccaggactgatccagaa

SEQ ID NO: 173 - DNA, 39 bp, Sus scrofa; identical to SEQ ID NO: 165
  source 1..39: mol_type = other DNA

SEQ ID NO: 174 - DNA, 39 bp, Sus scrofa; identical to SEQ ID NO: 165
  source 1..39: mol_type = other DNA

SEQ ID NO: 175 - DNA, 37 bp, Sus scrofa; identical to SEQ ID NO: 164
  source 1..37: mol_type = other DNA

SEQ ID NO: 176 - DNA, 39 bp, Sus scrofa
  source 1..39: mol_type = other DNA
ctacttcaacctgagtcaggtgttgggactgatccagaa

SEQ ID NO: 177 - DNA, 45 bp, Sus scrofa
  source 1..45: mol_type = other DNA
ctacttcaacctaagccaggttgaagtgttgggactgatccagaa

SEQ ID NO: 178 - DNA, 39 bp, Sus scrofa; identical to SEQ ID NO: 165
  source 1..39: mol_type = other DNA

SEQ ID NO: 179 - DNA, 41 bp, Sus scrofa; identical to SEQ ID NO: 168
  source 1..41: mol_type = other DNA

SEQ ID NO: 180 - DNA, 38 bp, Sus scrofa
  source 1..38: mol_type = other DNA
ctacctcaacctgagccaggggtgggactgatccagaa

SEQ ID NO: 181 - DNA, 41 bp, Sus scrofa
  source 1..41: mol_type = other DNA
ctacttcaacctgagcctggtgtgttgggactgatccagaa

SEQ ID NO: 182 - DNA, 39 bp, Sus scrofa; identical to SEQ ID NO: 165
  source 1..39: mol_type = other DNA

SEQ ID NO: 183 - DNA, 39 bp, Sus scrofa; identical to SEQ ID NO: 165
  source 1..39: mol_type = other DNA

SEQ ID NO: 184 - DNA, 38 bp, Sus scrofa
  source 1..38: mol_type = other DNA
ctacttcaacctgagccaggtctgggactgatccagaa

SEQ ID NO: 185 - DNA, 16 bp, Sus scrofa
  source 1..16: mol_type = other DNA
tgggactgatccagaa

SEQ ID NO: 186 - DNA, 45 bp, Sus scrofa
  source 1..45: mol_type = other DNA
ctacttcaacctgagccaggttgaagtgttgggactgatccagaa

SEQ ID NO: 187 - DNA, 45 bp, Sus scrofa; identical to SEQ ID NO: 186
  source 1..45: mol_type = other DNA

SEQ ID NO: 188 - DNA, 39 bp, Sus scrofa; identical to SEQ ID NO: 165
  source 1..39: mol_type = other DNA

SEQ ID NO: 189 - DNA, 39 bp, Sus scrofa; identical to SEQ ID NO: 165
  source 1..39: mol_type = other DNA

SEQ ID NO: 190 - DNA, 37 bp, Sus scrofa; identical to SEQ ID NO: 164
  source 1..37: mol_type = other DNA

SEQ ID NO: 191 - DNA, 37 bp, Sus scrofa; identical to SEQ ID NO: 164
  source 1..37: mol_type = other DNA

SEQ ID NO: 192 - DNA, 41 bp, Sus scrofa
  source 1..41: mol_type = other DNA
ctacttcaacctgagccaggtgtgttgggactgatcaataa

SEQ ID NO: 193 - DNA, 38 bp, Sus scrofa
  source 1..38: mol_type = other DNA
ctacttcaacctgagccagtgttgggactgatccagaa

SEQ ID NO: 194 - DNA, 39 bp, Sus scrofa; identical to SEQ ID NO: 165
  source 1..39: mol_type = other DNA

SEQ ID NO: 195 - DNA, 42 bp, Sus scrofa
  source 1..42: mol_type = other DNA
ctacttcaacctgagccaggcggggttgggactgatccagaa

SEQ ID NO: 196 - DNA, 39 bp, Sus scrofa; identical to SEQ ID NO: 165
  source 1..39: mol_type = other DNA

SEQ ID NO: 197 - DNA, 37 bp, Sus scrofa; identical to SEQ ID NO: 164
  source 1..37: mol_type = other DNA

SEQ ID NO: 198 - DNA, 41 bp, Sus scrofa; identical to SEQ ID NO: 168
  source 1..41: mol_type = other DNA

SEQ ID NO: 199 - DNA, 21 bp, Sus scrofa
  source 1..21: mol_type = other DNA
ctacttcaacctgagccagaa

SEQ ID NO: 200 - DNA, 51 bp, Sus scrofa
  source 1..51: mol_type = other DNA
atccagaatcgtcgacaagggccagaggccccgggcaccggggagccaaga

SEQ ID NO: 201 - DNA, 44 bp, Sus scrofa
  source 1..44: mol_type = other DNA
atccagaatcgtcgacaagggccccgggcaccggggagccaaga

SEQ ID NO: 202 - DNA, 44 bp, Sus scrofa; identical to SEQ ID NO: 201
  source 1..44: mol_type = other DNA

SEQ ID NO: 203 - DNA, 50 bp, Sus scrofa
  source 1..50: mol_type = other DNA
atccagaatcgtcgacgacgcgagaagccccgggcaccggggagccaaga

SEQ ID NO: 204 - DNA, 40 bp, Sus scrofa
  source 1..40: mol_type = other DNA
atccagaatcgtcgaggccccgggcaccggggagccaaga